European Patent Application EP 4 180 460 A1, published May 17, 2023. Title: SYSTEM AND METHOD FOR EDITING NUCLEIC ACID. Applicant: INSTITUTE OF ZOOLOGY, CHINESE ACADEMY OF SCIENCES; BEIJING INSTITUTE FOR STEM CELL AND REGENERATIVE MEDICINE. The sequence listing filed with the application follows.

SEQUENCE LISTING (84 sequences)

SEQ ID NO: 1 - protein, 1368 aa, artificial [sequence omitted]

SEQ ID NO: 2 - protein, 236 aa, artificial
  mCherry
MVSKGEEDNMAIIKEFMRFKVHMEGSVNGHEFEIEGEGEGRPYEGTQTAKLKVTKGGPLPFAWDILSPQFMYGSKAYVKHPADIPDYLKLSFPEGFKWERVMNFEDGGVVTVTQDSSLQDGEFIYKVKLRGTNFPSDGPVMQKKTMGWEASSERMYPEDGALKGEIKQRLKLKDGGHYDAEVKTTYKAKKPVQLPGAYNVNIKLDITSHNEDYTIVEQYERAEGRHSTGGMDELYK

SEQ ID NO: 3 - DNA, 76 bp, artificial
  gRNA without guide sequence
gttttagagctagaaatagcaagttaaaataaggctagtccgttatcaacttgaaaaagtggcaccgagtcggtgc

SEQ ID NO: 4 - protein, 722 aa, artificial
  MLV RT
MSETPGTSESATPESSGGSSGGSSTLNIEDEYRLHETSKEPDVSLGSTWLSDFPQAWAETGGMGLAVRQAPLIIPLKATSTPVSIKQYPMSQEARLGIKPHIQRLLDQGILVPCQSPWNTPLLPVKKPGTNDYRPVQDLREVNKRVEDIHPTVPNPYNLLSGLPPSHQWYTVLDLKDAFFCLRLHPTSQPLFAFEWRDPEMGISGQLTWTRLPQGFKNSPTLFNEALHRDLADFRIQHPDLILLQYVDDLLLAATSELDCQQGTRALLQTLGNLGYRASAKKAQICQKQVKYLGYLLKEGQRWLTEARKETVMGQPTPKTPRQLREFLGKAGFCRLFIPGFAEMAAPLYPLTKPGTLFNWGPDQQKAYQEIKQALLTAPALGLPDLTKPFELFVDEKQGYAKGVLTQKLGPWRRPVAYLSKKLDPVAAGWPPCLRMVAAIAVLTKDAGKLTMGQPLVILAPHAVEALVKQPPDRWLSNARMTHYQALLLDTDRVQFGPVVALNPATLLPLPEEGLQHNCLDILAEAHGTRPDLTDQPLPDADHTWYTDGSSLLQEGQRKAGAAVTTETEVIWAKALPAGTSAQRAELIALTQALKMAEGKKLNVYTDSRYAFATAHIHGEIYRRRGWLTSEGKEIKNKDEILALLKALFLPKRLSIIHCPGHQKGHSAEARGNRMADQAARKAAITETPDTSTLLIENSSPSGGSKRTADGSEFEPKKKRKV

SEQ ID NO: 5 - DNA, 24 bp, artificial
  Gapdh-gRNA-F
ccggagagagagaccctcactgct

SEQ ID NO: 6 - DNA, 24 bp, artificial
  Gapdh-gRNA-R
aaacagcagtgagggtctctctct

SEQ ID NO: 7 - DNA, 96 bp, artificial
  Gapdh-gRNA
agagagagaccctcactgctgttttagagctagaaatagcaagttaaaataaggctagtccgttatcaacttgaaaaagtggcaccgagtcggtgc

SEQ ID NO: 8 - DNA, 24 bp, artificial
  Actb-gRNA-F
ccggatcccccaaagttcacaatg

SEQ ID NO: 9 - DNA, 24 bp, artificial
  Actb-gRNA-R
aaaccattgtgaactttgggggat

SEQ ID NO: 10 - DNA, 96 bp, artificial
  Actb-gRNA
atcccccaaagttcacaatggttttagagctagaaatagcaagttaaaataaggctagtccgttatcaacttgaaaaagtggcaccgagtcggtgc

SEQ ID NO: 11 - DNA, 24 bp, artificial
  GapdhRC-gRNA-F
ccggtagcgttgacccgaccccaa

SEQ ID NO: 12 - DNA, 24 bp, artificial
  GapdhRC-gRNA-R
aaacttggggtcgggtcaacgcta

SEQ ID NO: 13 - DNA, 96 bp, artificial
  GapdhRC-gRNA
tagcgttgacccgaccccaagttttagagctagaaatagcaagttaaaataaggctagtccgttatcaacttgaaaaagtggcaccgagtcggtgc

SEQ ID NO: 14 - DNA, 24 bp, artificial
  GapdhRT-gRNA-F
ccgggtaagcacacgtgcaaagtg

SEQ ID NO: 15 - DNA, 24 bp, artificial
  GapdhRT-gRNA-R
aaaccactttgcacgtgtgcttac

SEQ ID NO: 16 - DNA, 96 bp, artificial
  GapdhRT-gRNA
gtaagcacacgtgcaaagtggttttagagctagaaatagcaagttaaaataaggctagtccgttatcaacttgaaaaagtggcaccgagtcggtgc

SEQ ID NO: 17 - DNA, 24 bp, artificial
  spacerA-gRNA-F
ccgggagatcgagtgccgcatcac

SEQ ID NO: 18 - DNA, 24 bp, artificial
  spacerA-gRNA-R
aaacgtgatgcggcactcgatctc

SEQ ID NO: 19 - DNA, 96 bp, artificial
  spacerA-gRNA
gagatcgagtgccgcatcacgttttagagctagaaatagcaagttaaaataaggctagtccgttatcaacttgaaaaagtggcaccgagtcggtgc

SEQ ID NO: 20 - DNA, 24 bp, artificial
  spacerK-gRNA-F
ccgggtcgccctcgaacttcacct

SEQ ID NO: 21 - DNA, 24 bp, artificial
  spacerK-gRNA-R
aaacaggtgaagttcgagggcgac

SEQ ID NO: 22 - DNA, 96 bp, artificial
  spacerK-gRNA
gtcgccctcgaacttcacctgttttagagctagaaatagcaagttaaaataaggctagtccgttatcaacttgaaaaagtggcaccgagtcggtgc

SEQ ID NO: 23 - DNA, 65 bp, artificial
  Gapdh-pegA-F
aaagtggcaccgagtcggtgcagcaagagcacaagaggaagagagagaccctcactatgcggcac

SEQ ID NO: 24 - DNA, 62 bp, artificial
  Gapdh-pegA-R
acagctatgaccatgattacgccaagcttaaaaaaaatcgagtgccgcatagtgagggtctc

SEQ ID NO: 25 - DNA, 144 bp, artificial
  Gapdh-pegA
gagatcgagtgccgcatcacgttttagagctagaaatagcaagttaaaataaggctagtccgttatcaacttgaaaaagtggcaccgagtcggtgcagcaagagcacaagaggaagagagagaccctcactatgcggcactcga

SEQ ID NO: 26 - DNA, 56 bp, artificial
  Gapdh-pegK-F
aaagtggcaccgagtcggtgctggtgggggactgagtgtggcagggactccccagc

SEQ ID NO: 27 - DNA, 60 bp, artificial
  Gapdh-pegK-R
gaccatgattacgccaagcttaaaaaaaaccctcgaacttcagctggggagtccctgcca

SEQ ID NO: 28 - DNA, 144 bp, artificial
  Gapdh-pegK
gtcgccctcgaacttcacctgttttagagctagaaatagcaagttaaaataaggctagtccgttatcaacttgaaaaagtggcaccgagtcggtgctggtgggggactgagtgtggcagggactccccagctgaagttcgaggg

SEQ ID NO: 29 - DNA, 62 bp, artificial
  Actb-pegA-F
aaagtggcaccgagtcggtgccagtcggttggagcgagcatcccccaaagttcacaatgcgg

SEQ ID NO: 30 - DNA, 66 bp, artificial
  Actb-pegA-R
acagctatgaccatgattacgccaagcttaaaaaaaatcgagtgccgcattgtgaactttggggga

SEQ ID NO: 31 - DNA, 144 bp, artificial
  Actb-pegA
gagatcgagtgccgcatcacgttttagagctagaaatagcaagttaaaataaggctagtccgttatcaacttgaaaaagtggcaccgagtcggtgccagtcggttggagcgagcatcccccaaagttcacaatgcggcactcga

SEQ ID NO: 32 - DNA, 66 bp, artificial
  Actb-pegK-F
aaagtggcaccgagtcggtgcaaacaacaatgtgcaatcaaagtcctcggccacattgaagttcga

SEQ ID NO: 33 - DNA, 63 bp, artificial
  Actb-pegK-R
acagctatgaccatgattacgccaagcttaaaaaaaaccctcgaacttcaatgtggccgagga

SEQ ID NO: 34 - DNA, 144 bp, artificial
  Actb-pegK
gtcgccctcgaacttcacctgttttagagctagaaatagcaagttaaaataaggctagtccgttatcaacttgaaaaagtggcaccgagtcggtgcaaacaacaatgtgcaatcaaagtcctcggccacattgaagttcgaggg

SEQ ID NO: 35 - DNA, 60 bp, artificial
  GapdhRC-pegRNA-F
aagtggcaccgagtcggtgctttacagcctggcctttggagatcgagtgccgcatgggtc

SEQ ID NO: 36 - DNA, 65 bp, artificial
  GapdhRC-pegRNA-R
aacagctatgaccatgattacgccaagcttaaaaaaaattgacccgacccatgcggcactcgatc

SEQ ID NO: 37 - DNA, 143 bp, artificial
  GapdhRC-pegRNA
tagcgttgacccgaccccaagttttagagctagaaatagcaagttaaaataaggctagtccgttatcaacttgaaaaagtggcaccgagtcggtgctttacagcctggcctttggagatcgagtgccgcatgggtcgggtcaa

SEQ ID NO: 38 - DNA, 61 bp, artificial
  GapdhRT-pegRNA-F
aagtggcaccgagtcggtgcgttactcccgggcctcacgtcgccctcgaacttcatttgca

SEQ ID NO: 39 - DNA, 68 bp, artificial
  GapdhRT-pegRNA-R
aacagctatgaccatgattacgccaagcttaaaaaaaagcacacgtgcaaatgaagttcgagggcgac

SEQ ID NO: 40 - DNA, 144 bp, artificial
  GapdhRT-pegRNA
gtaagcacacgtgcaaagtggttttagagctagaaatagcaagttaaaataaggctagtccgttatcaacttgaaaaagtggcaccgagtcggtgcgttactcccgggcctcacgtcgccctcgaacttcatttgcacgtgtgc

SEQ ID NO: 41 - DNA, 59 bp, artificial
  GapdhRC-pegA-F
aagtggcaccgagtcggtgcgcccttcccctgccagcctagcgttgacccgacccatgc

SEQ ID NO: 42 - DNA, 67 bp, artificial
  GapdhRC-pegA-R
acagctatgaccatgattacgccaagcttaaaaaaaatcgagtgccgcatgggtcgggtcaacgcta

SEQ ID NO: 43 - DNA, 144 bp, artificial
  GapdhRC-pegA
gagatcgagtgccgcatcacgttttagagctagaaatagcaagttaaaataaggctagtccgttatcaacttgaaaaagtggcaccgagtcggtgcgcccttcccctgccagcctagcgttgacccgacccatgcggcactcga

SEQ ID NO: 44 - DNA, 60 bp, artificial
  GapdhRT-pegK-F
aagtggcaccgagtcggtgctacttttgtctccactaggtaagcacacgtgcaaatgaag

SEQ ID NO: 45 - DNA, 71 bp, artificial
  GapdhRT-pegK-R
aacagctatgaccatgattacgccaagcttaaaaaaaaccctcgaacttcatttgcacgtgtgcttaccta

SEQ ID NO: 46 - DNA, 144 bp, artificial
  GapdhRT-pegK
gtcgccctcgaacttcacctgttttagagctagaaatagcaagttaaaataaggctagtccgttatcaacttgaaaaagtggcaccgagtcggtgctacttttgtctccactaggtaagcacacgtgcaaatgaagttcgaggg

SEQ ID NO: 47 - DNA, 1447 bp, artificial
  IRES-EGFP
ccggtgatgcggcactcgatctcgaattccccctctccctcccccccccctaacgttactggccgaagccgcttggaataaggccggtgtgcgtttgtctatatgttattttccaccatattgccgtcttttggcaatgtgagggcccggaaacctggccctgtcttcttgacgagcattcctaggggtctttcccctctcgccaaaggaatgcaaggtctgttgaatgtcgtgaaggaagcagttcctctggaagcttcttgaagacaaacaacgtctgtagcgaccctttgcaggcagcggaaccccccacctggcgacaggtgcctctgcggccaaaagccacgtgtataagatacacctgcaaaggcggcacaaccccagtgccacgttgtgagttggatagttgtggaaagagtcaaatggctctcctcaagcgtattcaacaaggggctgaaggatgcccagaaggtaccccattgtatgggatctgatctggggcctcggtgcacatgctttacatgtgtttagtcgaggttaaaaaaacgtctaggccccccgaaccacggggacgtggttttcctttgaaaaacacgatgataatatggccacaacgctcggtttaaaaagcttctatgcctgaataggtgaccggaggtcggcacctttcctttgcaattactgaccctatgaatacaggatctatggtgagcaagggcgaggagctgttcaccggggtggtgcccatcctggtcgagctggacggcgacgtaaacggccacaagttcagcgtgtccggcgagggcgagggcgatgccacctacggcaagctgaccctgaagttcatctgcactacggggaaactgcccgtgccctggcccaccctcgtgaccaccctgacctacggcgtgcagtgcttcagccgctaccccgaccacatgaagcagcacgacttcttcaagtccgccatgcccgaaggctacgtccaggagcgcaccatcttcttcaaggacgacggcaactacaagacccgcgctgaagtcaaattcgagggcgacaccctggtgaaccgcatcgagctgaagggcatcgacttcaaggaggacggcaacatcctggggcacaagctggagtacaactacaacagccacaacgtctatatcatggccgacaagcagaagaacggcatcaaggtgaacttcaagatccgccacaacatcgaggacggcagcgtgcagctcgccgaccactaccagcagaacacccccatcggcgacggccccgtgctgctgcccgacaaccactacctgagcacccagtccgccctgagcaaagaccccaacgagaagcgcgatcacatggtcctgctggagttcgtgaccgccgccgggatcactctcggcatggacgagctgtacaagtaagtcgccctcgaacttcacctcgg

SEQ ID NO: 48 - DNA, 4259 bp, artificial
  Gene fragment comprising T2A-EGFP
ccggtgatgcggcactcgatctccaaaggccaggctgtaaatgtcaccgggaggattgggtgtctgggcgcctcggggaacctgcccttctccccattccgtcttccggaaaccagatctcccaccgcaccctggtctgaggttaaatatagctgctgacctttctgtagctgggggcctgggctggggctctctcccatcccttctccccacacacatgcacttacctgtgctcccactcctgatttctggaaaagagctaggaaggacaggcaacttggcaaatcaaagccctgggactagggggttaaaatacagcttcccctcttcccacccgccccagtctctgtcccttttgtaggagggacttagagaaggggtgggcttgccctgtccagttaatttctgacctttactcctgccctttgagtttgatgatgctgagtgtacaagcgttttctccctaaagggtgcagctgagctaggcagcagcaagcattcctggggtggcatagtggggtggtgaataccatgtacaaagcttgtgcccagactgtgggtggcagtgccccacatggccgcttctcctggaagggcttcgtatgactgggggtgttgggcagccctggagccttcagttgcagccatgccttaagccaggccagcctggcagggaagctcaagggagataaaattcaacctcttgggccctcctgggggtaaggagatgctgcattcgccctcttaatggggaggtggcctagggctgctcacatattctggaggagcctcccctcctcatgccttcttgcctcttgtctcttagatttggtcgtattgggcgcctggtcaccagggctgcttttaactctggtaaagtggatattgttgccatcaatgaccccttcattgacctcaactacatggtgagtgctacatggtgagccccaaagctggtgtgggaggagccacctggctgatgggcagccccttcataccctcacgtattcccccaggtttacatgttccaatatgattccacccatggcaaattccatggcaccgtcaaggctgagaacgggaagcttgtcatcaatggaaatcccatcaccatcttccaggagtgagtggaagacagaatggaagaaatgtgctttggggaggcaactaggatggtgtggctcccttgggtatatggtaaccttgtgtccctcaatatggtcctgtccccatctcccccccacccccataggcgagatccctccaaaatcaagtggggcgatgctggcgctgagtacgtcgtggagtccactggcgtcttcaccaccatggagaaggctggggtgagtgcaggagggcccgcgggaggggaagctgactcagccctgcaaaggcaggacccgggttcataactgtctgcttctctgctgtaggctcatttgcaggggggagccaaaagggtcatcatctctgccccctctgctgatgcccccatgttcgtcatgggtgtgaaccatgagaagtatgacaacagcctcaagatcatcaggtgaggaaggcagggcccgtggagaagcggccagcctggcaccctatggacacgctcccctgacttgcgccccgctccctctttctttgcagcaatgcctcctgcaccaccaactgcttagcacccctggccaaggtcatccatgacaactttggtatcgtggaaggactcatggtatgagagctggggaatgggactgaggctcccacctttctcatccaagactggctcctccctgccggggctgcgtgcaaccctggggttgggggttctggggactggctttcccataatttcctttcaaggtggggagggaggtagaggggtgatgtggggagtacgctgcagggcctcactccttttgcagaccacagtccatgccatcactgccacccagaagactgtggatggcccctccgggaaactgtggcgtgatggccgcggggctctccagaacatcatccctgcctctactggcgctgccaaggctgtgggcaaggtcatccctgagctgaacgggaagctcactggcatggccttccgtgtccccactgccaacgtgtcagtggtggacctgacctgccgtctagaaaaacctgccaaatatgatgacatcaagaaggtggtgaagcaggcgtcggagggccccctcaagggcatcctgggctacactgagcaccaggtggtctcctctgacttcaacagcgacacccactcctccacctttgacgctggggctggcattgccctcaacgaccactttgtcaagctcatttcctggtatgtggctggggccagagactggctcttaaaaagtgcagggtctggcgccctctggtggctggctcagaaaaagggccctgacaactcttttcatcttctaggtatgacaacgaatttggctacagcaacagggtggtggacctcatggcccacatggcctccaaggaggagggcagaggaagtcttctaacatgcggtgacgtggaggagaatcccggcccaatggtgagcaagggcgaggagctgttcaccggggtggtgcccatcctggtcgaactcgatggagatgtgaacggccacaagttcagcgtgtccggcgagggcgagggcgatgccacctacggcaagctgaccctgaagttcatctgcactacggggaaactgcccgtgccctggcccaccctcgtgaccaccctgacctacggcgtgcagtgcttcagccgctaccccgaccacatgaagcagcacgacttcttcaagtccgccatgccagagggatatgtgcaagagcgcaccatcttcttcaaggacgacggcaactacaagacccgcgctgaagtcaaattcgagggcgacaccctggtgaaccgcatcgagctgaagggcatcgacttcaaggaggacggcaacatcctggggcacaagctggagtacaactacaacagccacaacgtctatatcatggccgacaagcagaagaacggcatcaaggtgaacttcaagatccgccacaacatcgaggacggcagcgtgcagctcgccgaccactaccagcagaacacccccatcggcgacggccccgtgctgctgcccgacaaccactacctgagcacccagtccgccctgagcaaagaccccaacgagaagcgcgatcacatggtcctgctggagttcgtgaccgccgccgggatcactctcggcatggacgagctgtacaagtaagacccctggaccaccagccccagcaagagcacaagaggaagagagagaccctcactgctggggagtccctgccacactcagtcccccaccacactgaatctcccctcctcacagttgccatgtagaccccttgaagaggggaggggcctagggagccgcaccttgtcatgtaccatcaataaagtaccctgtgctcaaccagttacttgtcctgtcttattctagggtctggggcagaggggagggaagctgggcttgtgtcaaggtgagacattcttgctggggagggacctggtatgttctcctcagactgagggtagggcctccaaacagccttgcttgcttcgagaaccatttgcttcccgctcagacgtcttgagtgctacaggaagctggcaccactacttcagagaacaaggccttttcctctcctcgctccagtcctaggctatctgctgttggccaaacatggaagaagctattctgtgggcagccccagggaggctgacaggtggaggaagtcagggctcgcactgggctctgacgctgactggttagtggagctcagcctggagctgagctgcagcgggcaattccagcttggcctccgcagctgtgaggtcttgagcacgtgctctattgctttctgtgccctcgtgtcttatctgaggacatcgtggccagcccctaaggtcttcaagcaggattcatctaggtaaaccaagtacctaaaaccatgcccaaggcggtaaggactatataatgtttaaaaatcggtaaaaatgcccacctcgcatagttttgaggaagatgaactgagatgtgtcagggtgacttatttccatcatcgtccttaggggaacttgggtaggggcaaggcgtgtagctgggacctaggtccagacccctggctctgccactgaacggctcagttgctttgggcagttactcccgggcctcacgtcgccctcgaacttcacctcgg

SEQ ID NO: 49 - DNA, 23 bp, artificial
  SpacerA
gagatcgagtgccgcatcaccgg

SEQ ID NO: 50 - DNA, 23 bp, artificial
  SpacerK
gtcgccctcgaacttcacctcgg

SEQ ID NO: 51 - protein, 10 aa, artificial
  Linker
SGGSSGGSSG

SEQ ID NO: 52 - protein, 2099 aa, artificial
  Fusion protein
MDKKYSIGLDIGTNSVGWAVITDEYKVPSKKFKVLGNTDRHSIKKNLIGALLFDSGETAEATRLKRTARRRYTRRKNRICYLQEIFSNEMAKVDDSFFHRLEESFLVEEDKKHERHPIFGNIVDEVAYHEKYPTIYHLRKKLVDSTDKADLRLIYLALAHMIKFRGHFLIEGDLNPDNSDVDKLFIQLVQTYNQLFEENPINASGVDAKAILSARLSKSRRLENLIAQLPGEKKNGLFGNLIALSLGLTPNFKSNFDLAEDAKLQLSKDTYDDDLDNLLAQIGDQYADLFLAAKNLSDAILLSDILRVNTEITKAPLSASMIKRYDEHHQDLTLLKALVRQQLPEKYKEIFFDQSKNGYAGYIDGGASQEEFYKFIKPILEKMDGTEELLVKLNREDLLRKQRTFDNGSIPHQIHLGELHAILRRQEDFYPFLKDNREKIEKILTFRIPYYVGPLARGNSRFAWMTRKSEETITPWNFEEVVDKGASAQSFIERMTNFDKNLPNEKVLPKHSLLYEYFTVYNELTKVKYVTEGMRKPAFLSGEQKKAIVDLLFKTNRKVTVKQLKEDYFKKIECFDSVEISGVEDRFNASLGTYHDLLKIIKDKDFLDNEENEDILEDIVLTLTLFEDREMIEERLKTYAHLFDDKVMKQLKRRRYTGWGRLSRKLINGIRDKQSGKTILDFLKSDGFANRNFMQLIHDDSLTFKEDIQKAQVSGQGDSLHEHIANLAGSPAIKKGILQTVKVVDELVKVMGRHKPENIVIEMARENQTTQKGQKNSRERMKRIEEGIKELGSQILKEHPVENTQLQNEKLYLYYLQNGRDMYVDQELDINRLSDYDVDHIVPQSFLKDDSIDNKVLTRSDKNRGKSDNVPSEEVVKKMKNYWRQLLNAKLITQRKFDNLTKAERGGLSELDKAGFIKRQLVETRQITKHVAQILDSRMNTKYDENDKLIREVKVITLKSKLVSDFRKDFQFYKVREINNYHHAHDAYLNAVVGTALIKKYPKLESEFVYGDYKVYDVRKMIAKSEQEIGKATAKYFFYSNIMNFFKTEITLANGEIRKRPLIETNGETGEIVWDKGRDFATVRKVLSMPQVNIVKKTEVQTGGFSKESILPKRNSDKLIARKKDWDPKKYGGFDSPTVAYSVLVVAKVEKGKSKKLKSVKELLGITIMERSSFEKNPIDFLEAKGYKEVKKDLIIKLPKYSLFELENGRKRMLASAGELQKGNELALPSKYVNFLYLASHYEKLKGSPEDNEQKQLFVEQHKHYLDEIIEQISEFSKRVILADANLDKVLSAYNKHRDKPIREQAENIIHLFTLTNLGAPAAFKYFDTTIDRKRYTSTKEVLDATLIHQSITGLYETRIDLSQLGGDSGGSSGGSSGSETPGTSESATPESSGGSSGGSSTLNIEDEYRLHETSKEPDVSLGSTWLSDFPQAWAETGGMGLAVRQAPLIIPLKATSTPVSIKQYPMSQEARLGIKPHIQRLLDQGILVPCQSPWNTPLLPVKKPGTNDYRPVQDLREVNKRVEDIHPTVPNPYNLLSGLPPSHQWYTVLDLKDAFFCLRLHPTSQPLFAFEWRDPEMGISGQLTWTRLPQGFKNSPTLFNEALHRDLADFRIQHPDLILLQYVDDLLLAATSELDCQQGTRALLQTLGNLGYRASAKKAQICQKQVKYLGYLLKEGQRWLTEARKETVMGQPTPKTPRQLREFLGKAGFCRLFIPGFAEMAAPLYPLTKPGTLFNWGPDQQKAYQEIKQALLTAPALGLPDLTKPFELFVDEKQGYAKGVLTQKLGPWRRPVAYLSKKLDPVAAGWPPCLRMVAAIAVLTKDAGKLTMGQPLVILAPHAVEALVKQPPDRWLSNARMTHYQALLLDTDRVQFGPVVALNPATLLPLPEEGLQHNCLDILAEAHGTRPDLTDQPLPDADHTWYTDGSSLLQEGQRKAGAAVTTETEVIWAKALPAGTSAQRAELIALTQALKMAEGKKLNVYTDSRYAFATAHIHGEIYRRRGWLTSEGKEIKNKDEILALLKALFLPKRLSIIHCPGHQKGHSAEARGNRMADQAARKAAITETPDTSTLLIENSSPSGGSKRTADGSEFEPKKKRKV

SEQ ID NO: 53 - DNA, 24 bp, artificial
  sgACTB2-F
ccggccaccgcaaatgcttctagg

SEQ ID NO: 54 - DNA, 24 bp, artificial
  sgACTB2-R
aaaccctagaagcatttgcggtgg

SEQ ID NO: 55 - DNA, 96 bp, artificial
  sgACTB2
ccaccgcaaatgcttctagggttttagagctagaaatagcaagttaaaataaggctagtccgttatcaacttgaaaaagtggcaccgagtcggtgc

SEQ ID NO: 56 - DNA, 24 bp, artificial
  ACTB2-sgL-F
ccgggagctggacggcgacgtaaa

SEQ ID NO: 57 - DNA, 24 bp, artificial
  ACTB2-sgL-R
aaactttacgtcgccgtccagctc

SEQ ID NO: 58 - DNA, 96 bp, artificial
  ACTB2-sgL
gagctggacggcgacgtaaagttttagagctagaaatagcaagttaaaataaggctagtccgttatcaacttgaaaaagtggcaccgagtcggtgc

SEQ ID NO: 59 - DNA, 24 bp, artificial
  ACTB2-sgR-F
ccggcatgcccgaaggctacgtcc

SEQ ID NO: 60 - DNA, 24 bp, artificial
  ACTB2-sgR-R
aaacggacgtagccttcgggcatg

SEQ ID NO: 61 - DNA, 96 bp, artificial
  ACTB2-sgR
catgcccgaaggctacgtccgttttagagctagaaatagcaagttaaaataaggctagtccgttatcaacttgaaaaagtggcaccgagtcggtgc

SEQ ID NO: 62 - DNA, 60 bp, artificial
  ACTB2-pegL-F
aaagtggcaccgagtcggtgcggcccctccatcgtccaccgcaaatgcttcacgtcgccg

SEQ ID NO: 63 - DNA, 60 bp, artificial
  ACTB2-pegL-R
aacagctatgaccatgattacgccaagcttaaaaaaaagacggcgacgtgaagcatttgc

SEQ ID NO: 64 - DNA, 137 bp, artificial
  ACTB2-pegL
gagctggacggcgacgtaaagttttagagctagaaatagcaagttaaaataaggctagtccgttatcaacttgaaaaagtggcaccgagtcggtgcggcccctccatcgtccaccgcaaatgcttcacgtcgccgtc

SEQ ID NO: 65 - DNA, 58 bp, artificial
  ACTB2-pegR-F
aaagtggcaccgagtcggtgcggtgtaacgcaactaagtcatagtccgcctcgtagcc

SEQ ID NO: 66 - DNA, 63 bp, artificial
  ACTB2-pegR-R
aacagctatgaccatgattacgccaagcttaaaaaaaacgaaggctacgaggcggactatgac

SEQ ID NO: 67 - DNA, 137 bp, artificial
  ACTB2-pegR
catgcccgaaggctacgtccgttttagagctagaaatagcaagttaaaataaggctagtccgttatcaacttgaaaaagtggcaccgagtcggtgcggtgtaacgcaactaagtcatagtccgcctcgtagccttcg

SEQ ID NO: 68 - DNA, 18 bp, artificial
  GAPDH-P1
aaaagtgcagggtctggc

SEQ ID NO: 69 - DNA, 20 bp, artificial
  GAPDH-P2
acaccggccttattccaagc

SEQ ID NO: 70 - DNA, 22 bp, artificial
  GAPDH-P3
ccgaccactaccagcagaacac

SEQ ID NO: 71 - DNA, 25 bp, artificial
  GAPDH-P4
ccagaccctagaataagacaggaca

SEQ ID NO: 72 - DNA, 22 bp, artificial
  ACTB-P1
gggagctgtcacatccagggtc

SEQ ID NO: 73 - DNA, 22 bp, artificial
  ACTB-P2
aagacggcaatatggtggaaaa

SEQ ID NO: 74 - DNA, 20 bp, artificial
  ACTB-P3
ctgcccgacaaccactacct

SEQ ID NO: 75 - DNA, 22 bp, artificial
  ACTB-P4
ctaaggctgctcaatgtcaagg

SEQ ID NO: 76 - DNA, 22 bp, artificial
  ACTB2-P1
gggagctgtcacatccagggtc

SEQ ID NO: 77 - DNA, 22 bp, artificial
  ACTB2-P2
catctccatcgagttcgaccag

SEQ ID NO: 78 - DNA, 20 bp, artificial
  ACTB2-P3
ctgcccgacaaccactacct

SEQ ID NO: 79 - DNA, 22 bp, artificial
  ACTB2-P4
ctaaggctgctcaatgtcaagg

SEQ ID NO: 80 - DNA, 23 bp, artificial
  spacer L
gagctggacggcgacgtaaacgg

SEQ ID NO: 81 - DNA, 23 bp, artificial
  spacer R
catgcccgaaggctacgtccagg

SEQ ID NO: 82 - DNA, 771 bp, artificial
  T2A-EGFP
gagggcagaggaagtcttctaacatgcggtgacgtggaggagaatcccggcccagtgagcaagggcgaggagctgttcaccggggtggtgcccatcctggtcgaactcgatggagatgtgaacggccacaagttcagcgtgtccggcgagggcgagggcgatgccacctacggcaagctgaccctgaagttcatctgcactacggggaaactgcccgtgccctggcccaccctcgtgaccaccctgacctacggcgtgcagtgcttcagccgctaccccgaccacatgaagcagcacgacttcttcaagtccgccatgccagagggatatgtgcaagagcgcaccatcttcttcaaggacgacggcaactacaagacccgcgctgaagtcaaattcgagggcgacaccctggtgaaccgcatcgagctgaagggcatcgacttcaaggaggacggcaacatcctggggcacaagctggagtacaactacaacagccacaacgtctatatcatggccgacaagcagaagaacggcatcaaggtgaacttcaagatccgccacaacatcgaggacggcagcgtgcagctcgccgaccactaccagcagaacacccccatcggcgacggccccgtgctgctgcccgacaaccactacctgagcacccagtccgccctgagcaaagaccccaacgagaagcgcgatcacatggtcctgctggagttcgtgaccgccgccgggatcactctcggcatggacgagctgtacaagtaa

SEQ ID NO: 83 - DNA, 800 bp, artificial
  ACTB2 LHA
tggacctggctggccgggacctgactgactacctcatgaagatcctcaccgagcgcggctacagcttcaccaccacggccgagcgggaaatcgtgcgtgacattaaggagaagctgtgctacgtcgccctggacttcgagcaagagatggccacggctgcttccagctcctccctggagaagagctacgagctgcctgacggccaggtcatcaccattggcaatgagcggttccgctgccctgaggcactcttccagccttccttcctgggtgagtggagactgtctcccggctctgcctgacatgagggttacccctcggggctgtgctgtggaagctaagtcctgccctcatttccctctcaggcatggagtcctgtggcatccacgaaactaccttcaactccatcatgaagtgtgacgtggacatccgcaaagacctgtacgccaacacagtgctgtctggcggcaccaccatgtaccctggcattgccgacaggatgcagaaggagatcactgccctggcacccagcacaatgaagatcaaggtgggtgtctttcctgcctgagctgacctgggcaggtcggctgtggggtcctgtggtgtgtggggagctgtcacatccagggtcctcactgcctgtccccttccctcctcagatcattgctcctcctgagcgcaagtactccgtgtggatcggcggctccatcctggcctcgctgtccaccttccagcagatgtggatcagcaagcaggagtatgacgagtccggcccctccatcgtccaccgcaaatgcttc

SEQ ID NO: 84 - DNA, 800 bp, artificial
  ACTB2 RHA
aggcggactatgacttagttgcgttacaccctttcttgacaaaacctaacttgcgcagaaaacaagatgagattggcatggctttatttgttttttttgttttgttttggttttttttttttttttggcttgactcaggatttaaaaactggaacggtgaaggtgacagcagtcggttggagcgagcatcccccaaagttcacaatgtggccgaggactttgattgcacattgttgtttttttaatagtcattccaaatatgagatgcgttgttacaggaagtcccttgccatcctaaaagccaccccacttctctctaaggagaatggcccagtcctctcccaagtccacacaggggaggtgatagcattgctttcgtgtaaattatgtaatgcaaaatttttttaatcttcgccttaatacttttttattttgttttattttgaatgatgagccttcgtgcccccccttcccccttttttgtcccccaacttgagatgtatgaaggcttttggtctccctgggagtgggtggaggcagccagggcttacctgtacactgacttgagaccagttgaataaaagtgcacaccttaaaaatgaggccaagtgtgactttgtggtgtggctgggttgggggcagcagagggtgaaccctgcaggagggtgaaccctgcaaaagggtggggcagtgggggccaacttgtccttacccagagtgcaggtgtgtggagatccctcctgccttgacattgagcagccttagagggtgggggaggctcaggggtcaggtctctgttc